European Patent Specification EP 3 655 541 B1, published August 27, 2025. Title: IMPROVED METHOD AND KIT FOR THE GENERATION OF DNA LIBRARIES FOR MASSIVELY PARALLEL SEQUENCING. Applicant: MENARINI SILICON BIOSYSTEMS S.P.A. The sequence listing filed with the application follows.

SEQUENCE LISTING (75 sequences)

SEQ ID NO: 1 - DNA, 87 bp, Artificial Sequence
  LIB_IL_index D701
caagcagaagacggcatacgagatcgagtaatgtgactggagttcagacgtgtgctcttccgatctagtgggattcctgctgtcagt

SEQ ID NO: 2 - DNA, 87 bp, Artificial Sequence
  LIB_IL_index D702
caagcagaagacggcatacgagattctccggagtgactggagttcagacgtgtgctcttccgatctagtgggattcctgctgtcagt

SEQ ID NO: 3 - DNA, 87 bp, Artificial Sequence
  LIB_IL_index D703
caagcagaagacggcatacgagataatgagcggtgactggagttcagacgtgtgctcttccgatctagtgggattcctgctgtcagt

SEQ ID NO: 4 - DNA, 87 bp, Artificial Sequence
  LIB_IL_index D704
caagcagaagacggcatacgagatggaatctcgtgactggagttcagacgtgtgctcttccgatctagtgggattcctgctgtcagt

SEQ ID NO: 5 - DNA, 87 bp, Artificial Sequence
  LIB_IL_index D705
caagcagaagacggcatacgagatttctgaatgtgactggagttcagacgtgtgctcttccgatctagtgggattcctgctgtcagt

SEQ ID NO: 6 - DNA, 87 bp, Artificial Sequence
  LIB_IL_index D706
caagcagaagacggcatacgagatacgaattcgtgactggagttcagacgtgtgctcttccgatctagtgggattcctgctgtcagt

SEQ ID NO: 7 - DNA, 87 bp, Artificial Sequence
  LIB_IL_index D707
caagcagaagacggcatacgagatagcttcaggtgactggagttcagacgtgtgctcttccgatctagtgggattcctgctgtcagt

SEQ ID NO: 8 - DNA, 87 bp, Artificial Sequence
  LIB_IL_index D708
caagcagaagacggcatacgagatgcgcattagtgactggagttcagacgtgtgctcttccgatctagtgggattcctgctgtcagt

SEQ ID NO: 9 - DNA, 87 bp, Artificial Sequence
  LIB_IL_index D709
caagcagaagacggcatacgagatcatagccggtgactggagttcagacgtgtgctcttccgatctagtgggattcctgctgtcagt

SEQ ID NO: 10 - DNA, 87 bp, Artificial Sequence
  LIB_IL_index D710
caagcagaagacggcatacgagatttcgcggagtgactggagttcagacgtgtgctcttccgatctagtgggattcctgctgtcagt

SEQ ID NO: 11 - DNA, 87 bp, Artificial Sequence
  LIB_IL_index D711
caagcagaagacggcatacgagatgcgcgagagtgactggagttcagacgtgtgctcttccgatctagtgggattcctgctgtcagt

SEQ ID NO: 12 - DNA, 87 bp, Artificial Sequence
  LIB_IL_index D712
caagcagaagacggcatacgagatctatcgctgtgactggagttcagacgtgtgctcttccgatctagtgggattcctgctgtcagt

SEQ ID NO: 13 - DNA, 70 bp, Artificial Sequence
  LIB_IL_index D501
aatgatacggcgaccaccgagatctacactatagcctgctcaccgaagtgggattcctgctgtcagttaa

SEQ ID NO: 14 - DNA, 70 bp, Artificial Sequence
  LIB_IL_index D502
aatgatacggcgaccaccgagatctacacatagaggcgctcaccgaagtgggattcctgctgtcagttaa

SEQ ID NO: 15 - DNA, 70 bp, Artificial Sequence
  LIB_IL_index D503
aatgatacggcgaccaccgagatctacaccctatcctgctcaccgaagtgggattcctgctgtcagttaa

SEQ ID NO: 16 - DNA, 70 bp, Artificial Sequence
  LIB_IL_index D504
aatgatacggcgaccaccgagatctacacggctctgagctcaccgaagtgggattcctgctgtcagttaa

SEQ ID NO: 17 - DNA, 70 bp, Artificial Sequence
  LIB_IL_index D505
aatgatacggcgaccaccgagatctacacaggcgaaggctcaccgaagtgggattcctgctgtcagttaa

SEQ ID NO: 18 - DNA, 70 bp, Artificial Sequence
  LIB_IL_index D506
aatgatacggcgaccaccgagatctacactaatcttagctcaccgaagtgggattcctgctgtcagttaa

SEQ ID NO: 19 - DNA, 70 bp, Artificial Sequence
  LIB_IL_index D507
aatgatacggcgaccaccgagatctacaccaggacgtgctcaccgaagtgggattcctgctgtcagttaa

SEQ ID NO: 20 - DNA, 70 bp, Artificial Sequence
  LIB_IL_index D508
aatgatacggcgaccaccgagatctacacgtactgacgctcaccgaagtgggattcctgctgtcagttaa

SEQ ID NO: 21 - DNA, 23 bp, Artificial Sequence
  Adapter P5
aatgatacggcgaccaccgagat

SEQ ID NO: 22 - DNA, 21 bp, Artificial Sequence
  Adapter P7
caagcagaagacggcatacga

SEQ ID NO: 23 - DNA, 33 bp, Artificial Sequence
  Ampli1™ custom sequencing primer
gctcaccgaagtgggattcctgctgtcagttaa

SEQ ID NO: 24 - DNA, 26 bp, Artificial Sequence
  Custom primer index 2 A (i5) [LNA-5’]
  misc_feature 2: /note="locked nucleic acid"
  misc_feature 6: /note="locked nucleic acid"
  misc_feature 11: /note="locked nucleic acid"
acagcaggaatcccacttcggtgagc

SEQ ID NO: 25 - DNA, 26 bp, Artificial Sequence
  Custom primer index 2 A (i5) [LNA-3’]
  misc_feature 18: /note="locked nucleic acid"
  misc_feature 22: /note="locked nucleic acid"
  misc_feature 24: /note="locked nucleic acid"
acagcaggaatcccacttcggtgagc

SEQ ID NO: 26 - DNA, 33 bp, Artificial Sequence
  Custom primer index 2(i5)[RNA]
  misc_feature 3: /note="5-carbon sugar is ribose"
  misc_feature 5: /note="5-carbon sugar is ribose"
  misc_feature 7: /note="5-carbon sugar is ribose"
  misc_feature 8: /note="5-carbon sugar is ribose"
  misc_feature 11: /note="5-carbon sugar is ribose"
  misc_feature 12: /note="5-carbon sugar is ribose"
  misc_feature 15: /note="5-carbon sugar is ribose"
  misc_feature 17: /note="5-carbon sugar is ribose"
  misc_feature 21: /note="5-carbon sugar is ribose"
  misc_feature 22: /note="5-carbon sugar is ribose"
  misc_feature 23: /note="5-carbon sugar is ribose"
  misc_feature 26: /note="5-carbon sugar is ribose"
  misc_feature 29: /note="5-carbon sugar is ribose"
  misc_feature 30: /note="5-carbon sugar is ribose"
  misc_feature 31: /note="5-carbon sugar is ribose"
ttaactgacagcaggaatcccactacggagagc

SEQ ID NO: 27 - DNA, 93 bp, Artificial Sequence
  MAL_IL_index D701
caagcagaagacggcatacgagatcgagtaatgtgactggagttcagacgtgtgctcttccgatctgtgagtgatggttgaggtagtgtggag

SEQ ID NO: 28 - DNA, 93 bp, Artificial Sequence
  MAL_IL_index D702
caagcagaagacggcatacgagattctccggagtgactggagttcagacgtgtgctcttccgatctgtgagtgatggttgaggtagtgtggag

SEQ ID NO: 29 - DNA, 93 bp, Artificial Sequence
  MAL_IL_index D703
caagcagaagacggcatacgagataatgagcggtgactggagttcagacgtgtgctcttccgatctgtgagtgatggttgaggtagtgtggag

SEQ ID NO: 30 - DNA, 93 bp, Artificial Sequence
  MAL_IL_index D704
caagcagaagacggcatacgagatggaatctcgtgactggagttcagacgtgtgctcttccgatctgtgagtgatggttgaggtagtgtggag

SEQ ID NO: 31 - DNA, 93 bp, Artificial Sequence
  MAL_IL_index D705
caagcagaagacggcatacgagatttctgaatgtgactggagttcagacgtgtgctcttccgatctgtgagtgatggttgaggtagtgtggag

SEQ ID NO: 32 - DNA, 93 bp, Artificial Sequence
  MAL_IL_index D706
caagcagaagacggcatacgagatacgaattcgtgactggagttcagacgtgtgctcttccgatctgtgagtgatggttgaggtagtgtggag

SEQ ID NO: 33 - DNA, 93 bp, Artificial Sequence
  MAL_IL_index D707
caagcagaagacggcatacgagatagcttcaggtgactggagttcagacgtgtgctcttccgatctgtgagtgatggttgaggtagtgtggag

SEQ ID NO: 34 - DNA, 93 bp, Artificial Sequence
  MAL_IL_index D708
caagcagaagacggcatacgagatgcgcattagtgactggagttcagacgtgtgctcttccgatctgtgagtgatggttgaggtagtgtggag

SEQ ID NO: 35 - DNA, 93 bp, Artificial Sequence
  MAL_IL_index D709
caagcagaagacggcatacgagatcatagccggtgactggagttcagacgtgtgctcttccgatctgtgagtgatggttgaggtagtgtggag

SEQ ID NO: 36 - DNA, 93 bp, Artificial Sequence
  MAL_IL_index D710
caagcagaagacggcatacgagatttcgcggagtgactggagttcagacgtgtgctcttccgatctgtgagtgatggttgaggtagtgtggag

SEQ ID NO: 37 - DNA, 93 bp, Artificial Sequence
  MAL_IL_index D711
caagcagaagacggcatacgagatgcgcgagagtgactggagttcagacgtgtgctcttccgatctgtgagtgatggttgaggtagtgtggag

SEQ ID NO: 38 - DNA, 93 bp, Artificial Sequence
  MAL_IL_index D712
caagcagaagacggcatacgagatctatcgctgtgactggagttcagacgtgtgctcttccgatctgtgagtgatggttgaggtagtgtggag

SEQ ID NO: 39 - DNA, 64 bp, Artificial Sequence
  MAL_IL_index D501
aatgatacggcgaccaccgagatctacactatagcctgtgagtgatggttgaggtagtgtggag

SEQ ID NO: 40 - DNA, 64 bp, Artificial Sequence
  MAL_IL_index D502
aatgatacggcgaccaccgagatctacacatagaggcgtgagtgatggttgaggtagtgtggag

SEQ ID NO: 41 - DNA, 64 bp, Artificial Sequence
  MAL_IL_index D503
aatgatacggcgaccaccgagatctacaccctatcctgtgagtgatggttgaggtagtgtggag

SEQ ID NO: 42 - DNA, 64 bp, Artificial Sequence
  MAL_IL_index D504
aatgatacggcgaccaccgagatctacacggctctgagtgagtgatggttgaggtagtgtggag

SEQ ID NO: 43 - DNA, 64 bp, Artificial Sequence
  MAL_IL_index D505
aatgatacggcgaccaccgagatctacacaggcgaaggtgagtgatggttgaggtagtgtggag

SEQ ID NO: 44 - DNA, 64 bp, Artificial Sequence
  MAL_IL_index D506
aatgatacggcgaccaccgagatctacactaatcttagtgagtgatggttgaggtagtgtggag

SEQ ID NO: 45 - DNA, 64 bp, Artificial Sequence
  MAL_IL_index D507
aatgatacggcgaccaccgagatctacaccaggacgtgtgagtgatggttgaggtagtgtggag

SEQ ID NO: 46 - DNA, 64 bp, Artificial Sequence
  MAL_IL_index D508
aatgatacggcgaccaccgagatctacacgtactgacgtgagtgatggttgaggtagtgtggag

SEQ ID NO: 47 - DNA, 27 bp, Artificial Sequence
  Custom Read 1 primer
gtgagtgatggttgaggtagtgtggag

SEQ ID NO: 48 - DNA, 27 bp, Artificial Sequence
  Custom primer index 1 (i7)
ctccacactacctcaaccatcactcac

SEQ ID NO: 49 - DNA, 33 bp, Artificial Sequence; identical to SEQ ID NO: 23
  Custom primer read 2 (optional)

SEQ ID NO: 50 - DNA, 21 bp, Artificial Sequence
  LIB
agtgggattcctgctgtcagt

SEQ ID NO: 51 - DNA, 27 bp, Artificial Sequence
  MALBAC
gtgagtgatggttgaggtagtgtggag

SEQ ID NO: 52 - DNA, 65 bp, Artificial Sequence
  LIB_IL_v2_index D701
caagcagaagacggcatacgagatcgagtaatgctcaccgaagtgggattcctgctgtcagttaa

SEQ ID NO: 53 - DNA, 65 bp, Artificial Sequence
  LIB_IL_v2_index D702
caagcagaagacggcatacgagattctccggagctcaccgaagtgggattcctgctgtcagttaa

SEQ ID NO: 54 - DNA, 65 bp, Artificial Sequence
  LIB_IL_v2_index D703
caagcagaagacggcatacgagataatgagcggctcaccgaagtgggattcctgctgtcagttaa

SEQ ID NO: 55 - DNA, 65 bp, Artificial Sequence
  LIB_IL_v2_index D704
caagcagaagacggcatacgagatggaatctcgctcaccgaagtgggattcctgctgtcagttaa

SEQ ID NO: 56 - DNA, 65 bp, Artificial Sequence
  LIB_IL_v2_index D705
caagcagaagacggcatacgagatttctgaatgctcaccgaagtgggattcctgctgtcagttaa

SEQ ID NO: 57 - DNA, 65 bp, Artificial Sequence
  LIB_IL_v2_index D706
caagcagaagacggcatacgagatacgaattcgctcaccgaagtgggattcctgctgtcagttaa

SEQ ID NO: 58 - DNA, 65 bp, Artificial Sequence
  LIB_IL_v2_index D707
caagcagaagacggcatacgagatagcttcaggctcaccgaagtgggattcctgctgtcagttaa

SEQ ID NO: 59 - DNA, 65 bp, Artificial Sequence
  LIB_IL_v2_index D708
caagcagaagacggcatacgagatgcgcattagctcaccgaagtgggattcctgctgtcagttaa

SEQ ID NO: 60 - DNA, 65 bp, Artificial Sequence
  LIB_IL_v2_index D709
caagcagaagacggcatacgagatcatagccggctcaccgaagtgggattcctgctgtcagttaa

SEQ ID NO: 61 - DNA, 65 bp, Artificial Sequence
  LIB_IL_v2_index D710
caagcagaagacggcatacgagatttcgcggagctcaccgaagtgggattcctgctgtcagttaa

SEQ ID NO: 62 - DNA, 65 bp, Artificial Sequence
  LIB_IL_v2_index D711
caagcagaagacggcatacgagatgcgcgagagctcaccgaagtgggattcctgctgtcagttaa

SEQ ID NO: 63 - DNA, 65 bp, Artificial Sequence
  LIB_IL_v2_index D712
caagcagaagacggcatacgagatctatcgctgctcaccgaagtgggattcctgctgtcagttaa

SEQ ID NO: 64 - DNA, 59 bp, Artificial Sequence
  MAL_IL_v2_index D701
caagcagaagacggcatacgagatcgagtaatgtgagtgatggttgaggtagtgtggag

SEQ ID NO: 65 - DNA, 59 bp, Artificial Sequence
  MAL_IL_v2_index D702
caagcagaagacggcatacgagattctccggagtgagtgatggttgaggtagtgtggag

SEQ ID NO: 66 - DNA, 59 bp, Artificial Sequence
  MAL_IL_v2_index D703
caagcagaagacggcatacgagataatgagcggtgagtgatggttgaggtagtgtggag

SEQ ID NO: 67 - DNA, 59 bp, Artificial Sequence
  MAL_IL_v2_index D704
caagcagaagacggcatacgagatggaatctcgtgagtgatggttgaggtagtgtggag

SEQ ID NO: 68 - DNA, 59 bp, Artificial Sequence
  MAL_IL_v2_index D705
caagcagaagacggcatacgagatttctgaatgtgagtgatggttgaggtagtgtggag

SEQ ID NO: 69 - DNA, 59 bp, Artificial Sequence
  MAL_IL_v2_index D706
caagcagaagacggcatacgagatacgaattcgtgagtgatggttgaggtagtgtggag

SEQ ID NO: 70 - DNA, 59 bp, Artificial Sequence
  MAL_IL_v2_index D707
caagcagaagacggcatacgagatagcttcaggtgagtgatggttgaggtagtgtggag

SEQ ID NO: 71 - DNA, 59 bp, Artificial Sequence
  MAL_IL_v2_index D708
caagcagaagacggcatacgagatgcgcattagtgagtgatggttgaggtagtgtggag

SEQ ID NO: 72 - DNA, 59 bp, Artificial Sequence
  MAL_IL_v2_index D709
caagcagaagacggcatacgagatcatagccggtgagtgatggttgaggtagtgtggag

SEQ ID NO: 73 - DNA, 59 bp, Artificial Sequence
  MAL_IL_v2_index D710
caagcagaagacggcatacgagatttcgcggagtgagtgatggttgaggtagtgtggag

SEQ ID NO: 74 - DNA, 59 bp, Artificial Sequence
  MAL_IL_v2_index D711
caagcagaagacggcatacgagatgcgcgagagtgagtgatggttgaggtagtgtggag

SEQ ID NO: 75 - DNA, 59 bp, Artificial Sequence
  MAL_IL_v2_index D712
caagcagaagacggcatacgagatctatcgctgtgagtgatggttgaggtagtgtggag